European Patent Application EP 4 116 293 A2, published January 11, 2023. Title: Rho Kinase Inhibitors. Applicant: Kadmon Corporation LLC. Application to be assigned. The sequence listing filed with the application follows.

SEQUENCE LISTING (196 sequences)

SEQ ID NO: 1 - protein, 7 aa, Artificial Sequence
  Human antibody library
GFTFSWY

SEQ ID NO: 2 - protein, 7 aa, Artificial Sequence
  Human antibody library
IYPSGGA

SEQ ID NO: 3 - protein, 6 aa, Artificial Sequence
  Human antibody library
GNYFDY

SEQ ID NO: 4 - protein, 115 aa, Artificial Sequence
  Human antibody library
EVQLLESGGGLVQPGGSLRLSCAASGFTFSWYVMGWVRQAPGKGLEWVSSIYPSGGATNYADSVKGRFTISRDNSKNTLYLQMNSLRAEDTAVYYCARGNYFDYWGQGTLVTVSS

SEQ ID NO: 5 - protein, 11 aa, Artificial Sequence
  Human antibody library
QGDSLRSYYAS

SEQ ID NO: 6 - protein, 7 aa, Artificial Sequence
  Human antibody library
QDTNRPS

SEQ ID NO: 7 - protein, 9 aa, Artificial Sequence
  Human antibody library
QAWDSNTAV

SEQ ID NO: 8 - protein, 109 aa, Artificial Sequence
  Human antibody library
QSVLTQDPAVSVALGQTVRITCQGDSLRSYYASWYQQKPGQSPLVVIYQDTNRPSGIPERFSGSNSGNTATLTISETQAMDEADYYCQAWDSNTAVFGGGTKLTVLGQP

SEQ ID NO: 9 - protein, 7 aa, Artificial Sequence
  Human antibody library
GFTFSWY

SEQ ID NO: 10 - protein, 6 aa, Artificial Sequence
  Human antibody library
GSSGGF

SEQ ID NO: 11 - protein, 7 aa, Artificial Sequence
  Human antibody library
GLAAPRS

SEQ ID NO: 12 - protein, 116 aa, Artificial Sequence
  Human antibody library
EVQLLESGGGLVQPGGSLRLSCAASGFTFSWYIMLWVRQAPGKGLEWVSSIGSSGGFTDYADSVKGRFTISRDNSKNTLYLQMNSLRAEDTAVYYCARGLAAPRSWGRGTLVTVSS

SEQ ID NO: 13 - protein, 13 aa, Artificial Sequence
  Human antibody library
SGSTSNIGNNAVI

SEQ ID NO: 14 - protein, 7 aa, Artificial Sequence
  Human antibody library
YDDLLPS

SEQ ID NO: 15 - protein, 11 aa, Artificial Sequence
  Human antibody library
ASWDDNLNGPL

SEQ ID NO: 16 - protein, 113 aa, Artificial Sequence
  Human antibody library
QSALTQPPSVSEAPGQRVTISCSGSTSNIGNNAVIWYQQLPGKAPKLLIYYDDLLPSGVSDRFSGSKSGTSGSLAISGLQSEDEADYYCASWDDNLNGPLFGGGTKLTVLRQP

SEQ ID NO: 17 - protein, 13 aa, Artificial Sequence
  Human antibody library
SGSSSNIGTYPVN

SEQ ID NO: 18 - protein, 7 aa, Artificial Sequence
  Human antibody library
STDQRPS

SEQ ID NO: 19 - protein, 9 aa, Artificial Sequence
  Human antibody library
QAWDSSTVV

SEQ ID NO: 20 - protein, 111 aa, Artificial Sequence
  Human antibody library
QSALTQPPSASGTPGQRVTISCSGSSSNIGTYPVNWYQQLPGAAPKLLIYSTDQRPSGVPDRFSGSNSGNTATLTISGTQAMDEADYYCQAWDSSTVVFGGGTKLTVLGQP

SEQ ID NO: 21 - protein, 11 aa, Artificial Sequence
  Human antibody library
SGDKLGDEYAS

SEQ ID NO: 22 - protein, 7 aa, Artificial Sequence
  Human antibody library
QDNKRPS

SEQ ID NO: 23 - protein, 9 aa, Artificial Sequence
  Human antibody library
QAWDSSTVV

SEQ ID NO: 24 - protein, 109 aa, Artificial Sequence
  Human antibody library
QSALTQPPSVSVSPGQTASITCSGDKLGDEYASWYQQKPGQSPVLVIYQDNKRPSGIPERFSGSNSGNTATLTISGTQAMDEADYYCQAWDSSTVVFGGGTKLTVLGQP

SEQ ID NO: 25 - protein, 11 aa, Artificial Sequence
  Human antibody library
SGDNLRHEYSS

SEQ ID NO: 26 - protein, 7 aa, Artificial Sequence
  Human antibody library
QDSKRPS

SEQ ID NO: 27 - protein, 9 aa, Artificial Sequence
  Human antibody library
QAWGSSTVV

SEQ ID NO: 28 - protein, 109 aa, Artificial Sequence
  Human antibody library
QYELTQPPSVSVSPGQTASITCSGDNLRHEYSSWYQQRPGQSPVLVIYQDSKRPSGIPERFSGSNSGNTATLTISGTQALDEADYYCQAWGSSTVVFGGGTKLTVLRQP

SEQ ID NO: 29 - protein, 11 aa, Artificial Sequence
  Human antibody library
SGEKLGDEYAS

SEQ ID NO: 30 - protein, 7 aa, Artificial Sequence
  Human antibody library
QDNKRPS

SEQ ID NO: 31 - protein, 9 aa, Artificial Sequence
  Human antibody library
QAWDSSTLL

SEQ ID NO: 32 - protein, 109 aa, Artificial Sequence
  Human antibody library
QSVLTQPPSVSVSPGQTASITCSGEKLGDEYASWYQQKPGQSPVLVIYQDNKRPSGIPERFSGSNSGNTATLTISGTQAMDEADYYCQAWDSSTLLFGGGTKLTVLGQP

SEQ ID NO: 33 - protein, 11 aa, Artificial Sequence
  from human Fab library
SGEKLGDEYAS

SEQ ID NO: 34 - protein, 7 aa, Artificial Sequence
  from human Fab library
QDNKRPS

SEQ ID NO: 35 - protein, 9 aa, Artificial Sequence
  from human Fab library
QAWDSSTLL

SEQ ID NO: 36 - protein, 109 aa, Artificial Sequence
  from human Fab library
QSELTQPPSVSVSPGQTASITCSGEKLGDEYASWYQQKPGQSPVLVIYQDNKRPSGIPERFSGSNSGNTATLTISGTQAMDEADYYCQAWDSSTLLFGGGTKLTVLGQP

SEQ ID NO: 37 - protein, 11 aa, Artificial Sequence
  Human antibody library
TGDKLGDQFAS

SEQ ID NO: 38 - protein, 7 aa, Artificial Sequence
  Human antibody library
QNDKRPS

SEQ ID NO: 39 - protein, 9 aa, Artificial Sequence
  Human antibody library
QAWDFSSAL

SEQ ID NO: 40 - protein, 109 aa, Artificial Sequence
  Human antibody library
QYELTQPPSVSVSPGQTATITCTGDKLGDQFASWYQHKPGQSPILLIYQNDKRPSGIPDRFSGSDSGNTATLTISGTQAMDEAHYYCQAWDFSSALFGGGTKLTVLGQP

SEQ ID NO: 41 - protein, 11 aa, Artificial Sequence
  Human antibody library
SGQILGERSAS

SEQ ID NO: 42 - protein, 7 aa, Artificial Sequence
  Human antibody library
QSSQRPS

SEQ ID NO: 43 - protein, 8 aa, Artificial Sequence
  Human antibody library
QTWDTSIL

SEQ ID NO: 44 - protein, 108 aa, Artificial Sequence
  Human antibody library
QSALTQPPSVSVSPGHTATITCSGQILGERSASWYQQRPGQAPVLVLYQSSQRPSGIPERFSGSISGNTATLTISGAQSIDEADYYCQTWDTSILFGGGTKLTVLSQP

SEQ ID NO: 45 - protein, 11 aa, Artificial Sequence
  Human antibody library
SGDALGNNYAS

SEQ ID NO: 46 - protein, 7 aa, Artificial Sequence
  Human antibody library
QDTKRPS

SEQ ID NO: 47 - protein, 10 aa, Artificial Sequence
  Human antibody library
QTWDRNTPYV

SEQ ID NO: 48 - protein, 110 aa, Artificial Sequence
  Human antibody library
QSALTQPPSVSVSPGQTAIITCSGDALGNNYASWYQQKPGQSPVLVIYQDTKRPSGIPERFSGSSSGNTATLTISETQTMDEADYYCQTWDRNTPYVFGAGTKVTVLGQP

SEQ ID NO: 49 - protein, 13 aa, Artificial Sequence
  Human antibody library
SGSSSNIGTNTLN

SEQ ID NO: 50 - protein, 7 aa, Artificial Sequence
  Human antibody library
ANNQRPS

SEQ ID NO: 51 - protein, 11 aa, Artificial Sequence
  Human antibody library
ATWDDSLIGPV

SEQ ID NO: 52 - protein, 113 aa, Artificial Sequence
  Human antibody library
QSALTQPPSVSGTPGQRVTISCSGSSSNIGTNTLNWYQQLPGTAPKLLIYANNQRPSGVPDRFSGSRSGTSASLAISGLQSDDEADYYCATWDDSLIGPVFGGGTKLTVLGQP

SEQ ID NO: 53 - protein, 13 aa, Artificial Sequence
  from human Fab library
SGSTSNIGNNAVI

SEQ ID NO: 54 - protein, 7 aa, Artificial Sequence
  from human Fab library
YDDLLPS

SEQ ID NO: 55 - protein, 11 aa, Artificial Sequence
  from human Fab library
ASWDDNLNGPL

SEQ ID NO: 56 - protein, 113 aa, Artificial Sequence
  from human Fab library
QYELTQPPSVSEAPGQRVTISCSGSTSNIGNNAVIWYQQLPGKAPKLLIYYDDLLPSGVSDRFSGSKSGTSGSLAISGLQSEDEADYYCASWDDNLNGPLFGGGTKLTVLRQP

SEQ ID NO: 57 - protein, 13 aa, Artificial Sequence
  Human antibody library
SGSSSNLGSNTVN

SEQ ID NO: 58 - protein, 7 aa, Artificial Sequence
  Human antibody library
TNSQRPS

SEQ ID NO: 59 - protein, 11 aa, Artificial Sequence
  Human antibody library
AAWDDSLNGWV

SEQ ID NO: 60 - protein, 113 aa, Artificial Sequence
  Human antibody library
QSELTQPPSASGTPGQRVTISCSGSSSNLGSNTVNWYQQLPGTAPKLLIYTNSQRPSGVPDRFSGLQSGTSASLAISGLQSEDEADYYCAAWDDSLNGWVFGGGTKLTVLSQP

SEQ ID NO: 61 - protein, 13 aa, Artificial Sequence
  Human antibody library
SGSSSNIESNYVY

SEQ ID NO: 62 - protein, 7 aa, Artificial Sequence
  Human antibody library
TNNQRPS

SEQ ID NO: 63 - protein, 11 aa, Artificial Sequence
  Human antibody library
ASWDDSLSGVV

SEQ ID NO: 64 - protein, 113 aa, Artificial Sequence
  Human antibody library
QSVLTQPPSASGTPGQRVTISCSGSSSNIESNYVYWYQQLPGTAPKLLIYTNNQRPSGVPDRFSGSKSGTSASLAISGLRSEDEADYYCASWDDSLSGVVFGGGTKLTVLRQP

SEQ ID NO: 65 - protein, 14 aa, Artificial Sequence
  Human antibody library
TGSSNDIGSYDYVS

SEQ ID NO: 66 - protein, 7 aa, Artificial Sequence
  Human antibody library
DVNNRPS

SEQ ID NO: 67 - protein, 9 aa, Artificial Sequence
  Human antibody library
MSYTITALL

SEQ ID NO: 68 - protein, 112 aa, Artificial Sequence
  Human antibody library
QSELTQPDSVSGSPGQSITISCTGSSNDIGSYDYVSWYQQHPGRAPKFILYDVNNRPSGVADRFSGFKSGNTASLTISGLQPDDEADYFCMSYTITALLFGGGTRVTVLGQP

SEQ ID NO: 69 - protein, 14 aa, Artificial Sequence
  Human antibody library
TGSSHDIGSYDYVS

SEQ ID NO: 70 - protein, 7 aa, Artificial Sequence
  Human antibody library
DVNNRPS

SEQ ID NO: 71 - protein, 9 aa, Artificial Sequence
  Human antibody library
MSYTITTLL

SEQ ID NO: 72 - protein, 112 aa, Artificial Sequence
  Human antibody library
QSALTQPDSVSGSPGQSITISCTGSSHDIGSYDYVSWYQYHPGKAPKFILYDVNNRPSGVSDRFSGSKSGNTASLTISGLQPDDEADYFCMSYTITTLLFGTGTRVTVLSQP

SEQ ID NO: 73 - protein, 14 aa, Artificial Sequence
  Human antibody library
AGTSSDVGAYDYVS

SEQ ID NO: 74 - protein, 7 aa, Artificial Sequence
  Human antibody library
DVYNRPS

SEQ ID NO: 75 - protein, 9 aa, Artificial Sequence
  Human antibody library
MSYTITTLL

SEQ ID NO: 76 - protein, 112 aa, Artificial Sequence
  Human antibody library
QSALTQPASMSGSRGQSITISCAGTSSDVGAYDYVSWYKHLPGNAPKFILYDVYNRPSGVSDRFSGSKSGNTASLTISGLQPDDEADYFCMSYTITTLLFGTGTRVTVLSQP

SEQ ID NO: 77 - protein, 14 aa, Artificial Sequence
  Human antibody library
TGSSHDIGAYDYVS

SEQ ID NO: 78 - protein, 7 aa, Artificial Sequence
  Human antibody library
DVYNRPS

SEQ ID NO: 79 - protein, 9 aa, Artificial Sequence
  Human antibody library
MSYTITTLL

SEQ ID NO: 80 - protein, 112 aa, Artificial Sequence
  Human antibody library
QSVLTQPDSVSGSPGQSITISCTGSSHDIGAYDYVSWYKHLPGNAPKFILYDVYNRPSGVSDRFSGSKSGNTASLTISGLQPDDEADYFCMSYTITTLLFGTGTRVTVLSQP

SEQ ID NO: 81 - protein, 14 aa, Artificial Sequence
  from human Fab library
TGSSHDIGAYDYVS

SEQ ID NO: 82 - protein, 7 aa, Artificial Sequence
  from human Fab library
DVYNRPS

SEQ ID NO: 83 - protein, 9 aa, Artificial Sequence
  from human Fab library
MSYTITTLL

SEQ ID NO: 84 - protein, 112 aa, Artificial Sequence
  from human Fab library
QSVLTQPASVSGSPGQSITISCTGSSHDIGAYDYVSWYKHLPGNAPKFILYDVYNRPSGVSDRFSGSKSGNTASLTISGLQPDDEADYFCMSYTITTLLFGTGTRVTVLSQP

SEQ ID NO: 85 - protein, 14 aa, Artificial Sequence
  from human Fab library
TGSSHDIGAYDYVS

SEQ ID NO: 86 - protein, 7 aa, Artificial Sequence
  from human Fab library
DVYNRPS

SEQ ID NO: 87 - protein, 9 aa, Artificial Sequence
  from human Fab library
MSYTITTLL

SEQ ID NO: 88 - protein, 112 aa, Artificial Sequence
  from human Fab library
QSVLTQPYSVSGSPGQSITISCTGSSHDIGAYDYVSWYKHLPGNAPKFILYDVYNRPSGVSDRFSGSKSGNTASLTISGLQPDDEADYFCMSYTITTLLFGTGTRVTVLSQP

SEQ ID NO: 89 - protein, 14 aa, Artificial Sequence
  Human antibody library
TGSSHDIGAYDYVS

SEQ ID NO: 90 - protein, 7 aa, Artificial Sequence
  Human antibody library
DVYNRPS

SEQ ID NO: 91 - protein, 9 aa, Artificial Sequence
  Human antibody library
MSYTITTLL

SEQ ID NO: 92 - protein, 112 aa, Artificial Sequence
  Human antibody library
QSALTQPDSVSGSPGQSITISCTGSSHDIGAYDYVSWYKHLPGNAPKFILYDVYNRPSGVSDRFSGSKSGNTASLTISGLQPDDEADYFCMSYTITTLLFGTGTRVTVLSQP

SEQ ID NO: 93 - protein, 14 aa, Artificial Sequence
  from human Fab library
TGSSHDIGAYDYVS

SEQ ID NO: 94 - protein, 7 aa, Artificial Sequence
  from human Fab library
DVYNRPS

SEQ ID NO: 95 - protein, 9 aa, Artificial Sequence
  from human Fab library
MSYTITTLL

SEQ ID NO: 96 - protein, 112 aa, Artificial Sequence
  from human Fab library
QSELTQPDSVSGSPGQSITISCTGSSHDIGAYDYVSWYKHLPGNAPKFILYDVYNRPSGVSDRFSGSKSGNTASLTISGLQPDDEADYFCMSYTITTLLFGTGTRVTVLSQP

SEQ ID NO: 97 - protein, 12 aa, Artificial Sequence
  Human antibody library
RASQSVSSSYLA

SEQ ID NO: 98 - protein, 7 aa, Artificial Sequence
  Human antibody library
GASSRAT

SEQ ID NO: 99 - protein, 9 aa, Artificial Sequence
  Human antibody library
QQFDSSPPT

SEQ ID NO: 100 - protein, 109 aa, Artificial Sequence
  Human antibody library
DIQMTQSPGTLSLSPGERATLSCRASQSVSSSYLAWYQQKPGQAPRLLMYGASSRATGFPDRFSGSGSGTDFSLTISRLEPEDFAVYYCQQFDSSPPTFGGGTKVEIKR

SEQ ID NO: 101 - protein, 12 aa, Artificial Sequence
  Human antibody library
RASERISSNYLM

SEQ ID NO: 102 - protein, 7 aa, Artificial Sequence
  Human antibody library
GASIRAT

SEQ ID NO: 103 - protein, 9 aa, Artificial Sequence
  Human antibody library
QQYYSSPLT

SEQ ID NO: 104 - protein, 109 aa, Artificial Sequence
  Human antibody library
DIQMTQSPGTLSVLPGERATLSCRASERISSNYLMWYQQKPGQAPRLLMYGASIRATGIPDRFSGSESGTDFTLTISRVEPEDFAVYYCQQYYSSPLTFGGGTKVEMKR

SEQ ID NO: 105 - protein, 12 aa, Artificial Sequence
  Human antibody library
RASQSISSNYLA

SEQ ID NO: 106 - protein, 7 aa, Artificial Sequence
  Human antibody library
GASSRST

SEQ ID NO: 107 - protein, 9 aa, Artificial Sequence
  Human antibody library
QQFDTLPIT

SEQ ID NO: 108 - protein, 109 aa, Artificial Sequence
  Human antibody library
DIQMTQSPGTLSLSPGERATLSCRASQSISSNYLAWYQQRPGQAPRLLIYGASSRSTGTPDRFSGSGSGTDFTLTISRLEPEDFAIYYCQQFDTLPITFGQGTRLDIKR

SEQ ID NO: 109 - protein, 13 aa, Artificial Sequence
  Human antibody library
RASQSIRSSGYLS

SEQ ID NO: 110 - protein, 7 aa, Artificial Sequence
  Human antibody library
GASTRAT

SEQ ID NO: 111 - protein, 9 aa, Artificial Sequence
  Human antibody library
QQYGSSTIT

SEQ ID NO: 112 - protein, 110 aa, Artificial Sequence
  Human antibody library
DIQMTQSPATLSLSPGERATLSCRASQSIRSSGYLSWFQQKPGQAPRLLIYGASTRATGTPARFSGSGSGTDFTLTIDRLESEDFAVYFCQQYGSSTITFGQGTRLEIKR

SEQ ID NO: 113 - protein, 12 aa, Artificial Sequence
  Human antibody library
RASQSVSSNYLG

SEQ ID NO: 114 - protein, 7 aa, Artificial Sequence
  Human antibody library
GASSRAT

SEQ ID NO: 115 - protein, 9 aa, Artificial Sequence
  Human antibody library
QQFDNLPVT

SEQ ID NO: 116 - protein, 109 aa, Artificial Sequence
  Human antibody library
DIQMTQSPGTLSLSPGERATLSCRASQSVSSNYLGWYQQKPGQAPRLLIYGASSRATGIPDRFSGSGSGTDFTLTISRLEPEDFAVYYCQQFDNLPVTFGGGTKVEMKR

SEQ ID NO: 117 - protein, 12 aa, Artificial Sequence
  Human antibody library
RASQSVSSNYLA

SEQ ID NO: 118 - protein, 7 aa, Artificial Sequence
  Human antibody library
GASSRAT

SEQ ID NO: 119 - protein, 9 aa, Artificial Sequence
  Human antibody library
QQFDTSPLT

SEQ ID NO: 120 - protein, 109 aa, Artificial Sequence
  Human antibody library
DIQMTQSPGTLSLSPGERATLSCRASQSVSSNYLAWYQQKPGQAPRLLIYGASSRATGIPDRFSGSGSGTDFTLTISRLEPEDFAVYYCQQFDTSPLTIGGGTRVDIKR

SEQ ID NO: 121 - protein, 12 aa, Artificial Sequence
  Human antibody library
RASQSVSSNYLA

SEQ ID NO: 122 - protein, 7 aa, Artificial Sequence
  Human antibody library
GASSRAT

SEQ ID NO: 123 - protein, 9 aa, Artificial Sequence
  Human antibody library
QQFDSSPLS

SEQ ID NO: 124 - protein, 109 aa, Artificial Sequence
  Human antibody library
DIQMTQSPGTLSLSPGERATLSCRASQSVSSNYLAWYQQKPGQAPRLLIYGASSRATGIPDRFSGSGSGTDFSLTISRLEPEDSAVYYCQQFDSSPLSFGGGTKVEIKR

SEQ ID NO: 125 - protein, 12 aa, Artificial Sequence
  Human antibody library
RASQSVSSWYLA

SEQ ID NO: 126 - protein, 7 aa, Artificial Sequence
  Human antibody library
GASNRAT

SEQ ID NO: 127 - protein, 9 aa, Artificial Sequence
  Human antibody library
QQFDSSPLT

SEQ ID NO: 128 - protein, 109 aa, Artificial Sequence
  Human antibody library
DIQMTQSPGTLSLSPGERATLSCRASQSVSSWYLAWYQQKPGQAPRLLMYGASNRATGIPDRFSGSGSGTDFTLTISRLEPEDSAVYYCQQFDSSPLTIGGGTKVEIKR

SEQ ID NO: 129 - protein, 12 aa, Artificial Sequence
  Human antibody library
RASQNVGSSYLA

SEQ ID NO: 130 - protein, 7 aa, Artificial Sequence
  Human antibody library
GASSRAT

SEQ ID NO: 131 - protein, 9 aa, Artificial Sequence
  Human antibody library
QQFDSSPPT

SEQ ID NO: 132 - protein, 109 aa, Artificial Sequence
  Human antibody library
DIQMTQSPGTLSLSPGERATLSCRASQNVGSSYLAWYQQKPGQAPRLLMYGASSRATGFPDRFSGSGSGTDFSLTISRLEPEDFAVYYCQQFDSSPPTFGGGTKVEIKR

SEQ ID NO: 133 - protein, 12 aa, Artificial Sequence
  Human antibody library
RASQSVSSSYLA

SEQ ID NO: 134 - protein, 7 aa, Artificial Sequence
  Human antibody library
GASSRAT

SEQ ID NO: 135 - protein, 9 aa, Artificial Sequence
  Human antibody library
QQFDSSPPT

SEQ ID NO: 136 - protein, 109 aa, Artificial Sequence; identical to SEQ ID NO: 100
  Human antibody library

SEQ ID NO: 137 - protein, 12 aa, Artificial Sequence
  from human antibody library
RASQSVSSSYLA

SEQ ID NO: 138 - protein, 7 aa, Artificial Sequence
  from human antibody library
GASSRAT

SEQ ID NO: 139 - protein, 9 aa, Artificial Sequence
  from human antibody library
QQFDSSPPT

SEQ ID NO: 140 - protein, 109 aa, Artificial Sequence
  from human antibody library
DIQMTQSPGTLSLSPGERATLSCRASQSVSSSYLAWYQQKPGRAPRLLMYGASSRATGFPDRFSGSGSGTDFSLTISRLEPEDFAVYYCQQFDSSPPTFGGGTKVEIKR

SEQ ID NO: 141 - protein, 12 aa, Artificial Sequence
  Human antibody library
RASQSVSSSYLA

SEQ ID NO: 142 - protein, 7 aa, Artificial Sequence
  Human antibody library
GASSRAT

SEQ ID NO: 143 - protein, 10 aa, Artificial Sequence
  Human antibody library
QQFGSSPPYT

SEQ ID NO: 144 - protein, 110 aa, Artificial Sequence
  Human antibody library
DIQMTQSPGTLSLSPGERATLSCRASQSVSSSYLAWYQQKPGQAPRLLIYGASSRATGIPDRFSGSGSGTDYTLTINRLEPEDFAVYYCQQFGSSPPYTFGQGTKLEIKR

SEQ ID NO: 145 - protein, 12 aa, Artificial Sequence
  Human antibody library
RASQSVSSSYLA

SEQ ID NO: 146 - protein, 7 aa, Artificial Sequence
  Human antibody library
GASTRAT

SEQ ID NO: 147 - protein, 10 aa, Artificial Sequence
  Human antibody library
QQFDNWPPWT

SEQ ID NO: 148 - protein, 110 aa, Artificial Sequence
  Human antibody library
DIQMTQSPGTLSLSPGERATLSCRASQSVSSSYLAWYQQKPGQAPRLLIYGASTRATGIPPRFSGSGSGTEFTLTISSVQSEDFAIYYCQQFDNWPPWTFGQGTKVEIKR

SEQ ID NO: 149 - protein, 12 aa, Artificial Sequence
  Human antibody library
RASQSVSSNYFG

SEQ ID NO: 150 - protein, 7 aa, Artificial Sequence
  Human antibody library
GASSRAT

SEQ ID NO: 151 - protein, 9 aa, Artificial Sequence
  Human antibody library
QQFDSSPLT

SEQ ID NO: 152 - protein, 109 aa, Artificial Sequence
  Human antibody library
DIQMTQSPGTLSLSPGEGATLSCRASQSVSSNYFGWYQQKPGQAPRLLIYGASSRATGIPDRFSGSGSGTDFTLTISRLEPEDSAVYYCQQFDSSPLTFGGGTKVEIKR

SEQ ID NO: 153 - protein, 12 aa, Artificial Sequence
  from human antibody library
RASQSVSSNYLA

SEQ ID NO: 154 - protein, 7 aa, Artificial Sequence
  Human antibody library
GASSRAT

SEQ ID NO: 155 - protein, 9 aa, Artificial Sequence
  Human antibody library
QQFDSSPLS

SEQ ID NO: 156 - protein, 109 aa, Artificial Sequence; identical to SEQ ID NO: 124
  Human antibody library

SEQ ID NO: 157 - protein, 12 aa, Artificial Sequence
  Human antibody library
RASQSVSSNYLA

SEQ ID NO: 158 - protein, 7 aa, Artificial Sequence
  Human antibody library
GASTRAT

SEQ ID NO: 159 - protein, 9 aa, Artificial Sequence
  Human antibody library
QQFDSSPLS

SEQ ID NO: 160 - protein, 109 aa, Artificial Sequence
  Human antibody library
DIQMTQSPGTLSLSPGDRATLSCRASQSVSSNYLAWYQQKPGQAPRVLIYGASTRATGIPDRFTGSGSGTDFTLTISRLEPEDSAVYYCQQFDSSPLSFGGGTKVEIKR

SEQ ID NO: 161 - protein, 12 aa, Artificial Sequence
  Human antibody library
RASQSLNNNYLA

SEQ ID NO: 162 - protein, 7 aa, Artificial Sequence
  Human antibody library
GASTRAT

SEQ ID NO: 163 - protein, 9 aa, Artificial Sequence
  Human antibody library
QQFDSSPPT

SEQ ID NO: 164 - protein, 109 aa, Artificial Sequence
  Human antibody library
DIQMTQSPGTLSLSPGERATLSCRASQSLNNNYLAWYQQKPGQAPRLLMYGASTRATGIPARFSGSGSGTEFTLTISSLQSEDFAVYYCQQFDSSPPTFGGGTKVEIKR

SEQ ID NO: 165 - protein, 12 aa, Artificial Sequence
  Human antibody library
RASHSVSSDYLA

SEQ ID NO: 166 - protein, 7 aa, Artificial Sequence
  Human antibody library
GASSRAT

SEQ ID NO: 167 - protein, 9 aa, Artificial Sequence
  Human antibody library
QQFDSSPPT

SEQ ID NO: 168 - protein, 109 aa, Artificial Sequence
  Human antibody library
DIQMTQSPATLSLSPGERATLSCRASHSVSSDYLAWYQQKPGRAPRLLMYGASSRATGFPDRFSGSGSGTDFSLTISRLEPEDFAMYYCQQFDSSPPTFGGGTKVEIKR

SEQ ID NO: 169 - protein, 12 aa, Artificial Sequence
  from human antibody library
RASHSVSSDYLA

SEQ ID NO: 170 - protein, 7 aa, Artificial Sequence
  from human antibody library
GASSRAT

SEQ ID NO: 171 - protein, 9 aa, Artificial Sequence
  from human antibody library
QQFDSSPPT

SEQ ID NO: 172 - protein, 109 aa, Artificial Sequence
  from human antibody library
DIQMTQSPATLSVSPGERATLSCRASHSVSSDYLAWYQQKPGRAPRLLMYGASSRATGFPDRFSGSGSGTDFSLTISRLEPEDFAMYYCQQFDSSPPTFGGGTKVEIKR

SEQ ID NO: 173 - protein, 12 aa, Artificial Sequence
  Human antibody library
RASHSVSSDYLA

SEQ ID NO: 174 - protein, 7 aa, Artificial Sequence
  Human antibody library
GASSRAT

SEQ ID NO: 175 - protein, 9 aa, Artificial Sequence
  Human antibody library
QQFDSSPPT

SEQ ID NO: 176 - protein, 109 aa, Artificial Sequence
  Human antibody library
DIQMTQSPGTLSLSPGERATLSCRASHSVSSDYLAWYQQKPGRAPRLLMYGASSRATGFPDRFSGSGSGTDFSLTISRLEPEDFAVYYCQQFDSSPPTFGGGTKVEIKR

SEQ ID NO: 177 - protein, 12 aa, Artificial Sequence
  Human antibody library
RASHSVSSDYLA

SEQ ID NO: 178 - protein, 7 aa, Artificial Sequence
  Human antibody library
GASSRAT

SEQ ID NO: 179 - protein, 9 aa, Artificial Sequence
  Human antibody library
QQFDSSPPT

SEQ ID NO: 180 - protein, 111 aa, Artificial Sequence
  from human Fab library
IADIQMTQSPDTLSLSPGERATLSCRASHSVSSDYLAWYQQKPGRAPRLLMYGASSRATGFPDRFSGSGSGTDFSLTISRLEPEDFAVYYCQQFDSSPPTFGGGTKVEIKR

SEQ ID NO: 181 - protein, 12 aa, Artificial Sequence
  from human antibody library
RASHSVSSDYLA

SEQ ID NO: 182 - protein, 7 aa, Artificial Sequence
  from human antibody library
GASSRAT

SEQ ID NO: 183 - protein, 9 aa, Artificial Sequence
  from human antibody library
QQFDSSPPT

SEQ ID NO: 184 - protein, 109 aa, Artificial Sequence
  from human antibody library
DIQMTQSPDTLSLSPGERATLSCRASHSVSSDYLAWYQQKPGRAPRLLMYGASSRATGFPDRFSGSGSGTDFSLTISRLEPEDFAVYYCQQFDSSPPTFGGGTRIDIKR

SEQ ID NO: 185 - protein, 10 aa, Artificial Sequence
  consensus
  VARIANT (8)..(8): residue is V or I
  VARIANT (10)..(10): residue is G or L
GFTFSWYXMX

SEQ ID NO: 186 - protein, 17 aa, Artificial Sequence
  consensus
  VARIANT (3)..(3): residue is Y or G
  VARIANT (4)..(4): residue is P or S
  VARIANT (8)..(8): residue is A or F
  VARIANT (10)..(10): residue is N or D
SIXXSGGXTXYADSVKG

SEQ ID NO: 187 - protein, 11 aa, Artificial Sequence
  consensus
  VARIANT (1)..(1): residue is S Q or T
  VARIANT (3)..(3): residue is D E or Q
  VARIANT (4)..(4): residue is K S N I or A
  VARIANT (6)..(6): residue is G or R
  VARIANT (7)..(7): residue is D S H E or N
  VARIANT (8)..(8): residue is E Y Q R or N
  VARIANT (9)..(9): residue is Y F or S
  VARIANT (10)..(10): residue is A or S
XGXXLXXXXXS

SEQ ID NO: 188 - protein, 13 aa, Artificial Sequence
  consensus
  VARIANT (4)..(4): residue is S or T
  VARIANT (7)..(7): residue is I or L
  VARIANT (8)..(8): residue is E or G
  VARIANT (9)..(9): residue is T S or N
  VARIANT (10)..(10): residue is N or Y
  VARIANT (11)..(11): residue is T P A or Y
  VARIANT (12)..(12): residue is V or L
  VARIANT (13)..(13): residue is N I or Y
SGSXSNXXXXXXX

SEQ ID NO: 189 - protein, 14 aa, Artificial Sequence
  consensus
  VARIANT (1)..(1): residue is A or T
  VARIANT (3)..(3): residue is S or T
  VARIANT (5)..(5): residue is H S or N
  VARIANT (7)..(7): residue is I or V
  VARIANT (9)..(9): residue is S or A
XGXSXDXGXYDYVS

SEQ ID NO: 190 - protein, 7 aa, Artificial Sequence
  consensus
  VARIANT (1)..(1): residue is Q D T Y S or A
  VARIANT (2)..(2): residue is D N S T or V
  VARIANT (3)..(3): residue is D N S T or Y
  VARIANT (4)..(4): residue is Q K N or L
  VARIANT (5)..(5): residue is R or L
XXXXXPS

SEQ ID NO: 191 - protein, 10 aa, Artificial Sequence
  consensus
  VARIANT (2)..(2): residue is A or T
  VARIANT (4)..(4): residue is D or G
  VARIANT (5)..(5): residue is R or no amino acid
  VARIANT (6)..(6): residue is S F or N
  VARIANT (7)..(7): residue is S T or N
  VARIANT (8)..(8): residue is S T or P
  VARIANT (9)..(9): residue is A V L I or Y
  VARIANT (10)..(10): residue is V or L
QXWXXXXXXX

SEQ ID NO: 192 - protein, 11 aa, Artificial Sequence
  consensus
  VARIANT (2)..(2): residue is A S or T
  VARIANT (6)..(6): residue is N or S
  VARIANT (8)..(8): residue is N I or G
  VARIANT (9)..(9): residue is G or S
  VARIANT (10)..(10): residue is P W or V
  VARIANT (11)..(11): residue is V or L
AXWDDXLXXXX

SEQ ID NO: 193 - protein, 9 aa, Artificial Sequence
  consensus
  VARIANT (7)..(7): residue is A or T
MYSTITXLL

SEQ ID NO: 194 - protein, 13 aa, Artificial Sequence
  consensus
  VARIANT (4)..(4): residue is Q E or H
  VARIANT (5)..(5): residue is S R or N
  VARIANT (6)..(6): residue is V I or L
  VARIANT (7)..(7): residue is S R G or N
  VARIANT (8)..(8): residue is S or N
  VARIANT (9)..(9): residue is S N W or D
  VARIANT (10)..(10): residue is G or no amino acid
  VARIANT (12)..(12): residue is L or F
  VARIANT (13)..(13): residue is A G M or S
RASXXXXXXXYXX

SEQ ID NO: 195 - protein, 7 aa, Artificial Sequence
  consensus
  VARIANT (4)..(4): residue is S T I or N
GASXRAT

SEQ ID NO: 196 - protein, 10 aa, Artificial Sequence
  consensus
  VARIANT (3)..(3): residue is F or Y
  VARIANT (4)..(4): residue is D G or Y
  VARIANT (5)..(5): residue is S T or N
  VARIANT (6)..(6): residue is S L or W
  VARIANT (7)..(7): residue is P or no amino acid
  VARIANT (8)..(8): residue is P or T
  VARIANT (9)..(9): residue is L I V P W or Y
  VARIANT (10)..(10): residue is T or S
QQXXXXXXXX